European Patent Application EP 4 748 943 A1, published May 27, 2026. Title: CHIP, PREPARATION METHOD THEREFOR AND USE THEREOF. Applicant: GeneMind Biosciences Co., Ltd. Application EP. The sequence listing filed with the application follows.

SEQUENCE LISTING (14 sequences)

SEQ ID NO: 1 - DNA, 136 bp, Artificial Sequence
  source 1..136: mol_type = other DNA
aacgaaagtacttattgcaggtggtacggctggtctacactggactgcggaattctatgacgccagacatgttgcgaacnnnnnnnnnnnnnnnnnnnnnnnnnnnnnnnnagactgaaagtacgtgcattacatg

SEQ ID NO: 2 - DNA, 39 bp, Artificial Sequence
  source 1..39: mol_type = other DNA
aacgaaagtacttattgcaggtggtacggctggtctaca

SEQ ID NO: 3 - DNA, 40 bp, Artificial Sequence
  source 1..40: mol_type = other DNA
ctggactgcggaattctatgacgccagacatgttgcgaac

SEQ ID NO: 4 - DNA, 25 bp, Artificial Sequence
  source 1..25: mol_type = other DNA
agactgaaagtacgtgcattacatg

SEQ ID NO: 5 - DNA, 60 bp, Artificial Sequence
  source 1..60: mol_type = other DNA
ttttttttttaccacctgcaataagtactttcgttcatgtaatgcacgtactttcagtct

SEQ ID NO: 6 - DNA, 35 bp, Artificial Sequence
  source 1..35: mol_type = other DNA
ttttttttttcatgtaatgcacgtactttcagtct

SEQ ID NO: 7 - DNA, 94 bp, Artificial Sequence
  source 1..94: mol_type = other DNA
nbaaaaaaaaaaaaaaaaaaaaaaaaaaaaaaaaaaaaaaaaaaannnnnnnnnnaacgaaagtacttattgcaggtggtacggctggtctaca

SEQ ID NO: 8 - DNA, 35 bp, Artificial Sequence
  source 1..35: mol_type = other DNA
gagtggaactggatggtcgcaggtatctcgtcggg

SEQ ID NO: 9 - DNA, 25 bp, Artificial Sequence
  source 1..25: mol_type = other DNA
catgtaatgcacgtactttcagtct

SEQ ID NO: 10 - DNA, 32 bp, Artificial Sequence
  source 1..32: mol_type = other DNA
gacgagatacctgcgaccatccagttccactc

SEQ ID NO: 11 - DNA, 19 bp, Artificial Sequence
  source 1..19: mol_type = other DNA
ctgtctcttatacacatct

SEQ ID NO: 12 - DNA, 33 bp, Artificial Sequence
  source 1..33: mol_type = other DNA
tcgtcggcagcgtcagatgtgtataagagacag

SEQ ID NO: 13 - DNA, 25 bp, Artificial Sequence
  source 1..25: mol_type = other DNA
catgtaatgcacgtactttcagtct

SEQ ID NO: 14 - DNA, 33 bp, Artificial Sequence; identical to SEQ ID NO: 12
  source 1..33: mol_type = other DNA